European Patent Specification EP 3 230 477 B1, published January 17, 2024. Title: Methods for Capturing Nucleic Acids. Applicant: General Electric Company Nelson, John Li, Bing. Application PCT/US15/63468. The sequence listing filed with the application follows.

SEQUENCE LISTING (7 sequences)

SEQ ID NO: 1 - DNA, 25 bp, Artificial sequence
  Synthetic oliogonucleotide
catcattgatttagacactgaaaaa

SEQ ID NO: 2 - DNA, 20 bp, Artificial sequence
  Synthetic oligonucleotide
atcaatgatgtttttcagtg

SEQ ID NO: 3 - DNA, 19 bp, Artificial sequence
  Synthetic oligonucleotide
aggtaatggtgcagtaggt

SEQ ID NO: 4 - DNA, 43 bp, Artificial sequence
  Synthetic oligonucleotide
gcataatactaccagtctcctcagcaagctacgcattttcatt

SEQ ID NO: 5 - DNA, 44 bp, Artificial sequence
  Synthetic oliogonucleotide
tagaatagtcgcatacttcctcagcacatctcctcgaacttttt

SEQ ID NO: 6 - DNA, 17 bp, Artificial sequence
  Synthetic oligonucleotide
ccagctttcacacgaac

SEQ ID NO: 7 - DNA, 18 bp, Artificial sequence
  Synthetic oligonucleotide
ctaattcatcaacaatgc